European Patent Application EP 4 636 093 A1, published October 22, 2025. Title: TARGETING MAPK-ERK PATHWAY FOR ENHANCING NUCLEIC ACID DELIVERY. Applicant: Paul Ehrlich Institut. The sequence listing filed with the application follows.

SEQUENCE LISTING (4 sequences)

SEQ ID NO: 1 - DNA, 12150 bp, synthetic construct
  source 1..12150: mol_type = other DNA; note = pCMV-dR8.91
ttgattattgactagttattaatagtaatcaattacggggtcattagttcatagcccatatatggagttccgcgttacataacttacggtaaatggcccgcctggctgaccgcccaacgacccccgcccattgacgtcaataatgacgtatgttcccatagtaacgccaatagggactttccattgacgtcaatgggtggagtatttacggtaaactgcccacttggcagtacatcaagtgtatcatatgccaagtacgccccctattgacgtcaatgacggtaaatggcccgcctggcattatgcccagtacatgaccttatgggactttcctacttggcagtacatctacgtattagtcatcgctattaccatggtgatgcggttttggcagtacatcaatgggcgtggatagcggtttgactcacggggatttccaagtctccaccccattgacgtcaatgggagtttgttttggcaccaaaatcaacgggactttccaaaatgtcgtaacaactccgccccattgacgcaaatgggcggtaggcgtgtacggtgggaggtctatataagcagagctcgtttagtgaaccgtcagatcgcctggagacgccatccacgctgttttgacctccatagaagacaccgggaccgatccagcctccgcggccgggaacggtgcattggaacgcggattccccgtgccaagagtgacgtaagtaccgcctatagagtctataggcccacccccttggcttcttatgcgacggatcgatcccgtaataagcttcgaggtccgcggccggccgcgttgacgcgcacggcaagaggcgaggggcggcgactggtgagagatgggtgcgagagcgtcagtattaagcgggggagaattagatcgatgggaaaaaattcggttaaggccagggggaaagaaaaaatataaattaaaacatatagtatgggcaagcagggagctagaacgattcgcagttaatcctggcctgttagaaacatcagaaggctgtagacaaatactgggacagctacaaccatcccttcagacaggatcagaagaacttagatcattatataatacagtagcaaccctctattgtgtgcatcaaaggatagagataaaagacaccaaggaagctttagacaagatagaggaagagcaaaacaaaagtaagaaaaaagcacagcaagcagcagctgacacaggacacagcaatcaggtcagccaaaattaccctatagtgcagaacatccaggggcaaatggtacatcaggccatatcacctagaactttaaatgcatgggtaaaagtagtagaagagaaggctttcagcccagaagtgatacccatgttttcagcattatcagaaggagccaccccacaagatttaaacaccatgctaaacacagtggggggacatcaagcagccatgcaaatgttaaaagagaccatcaatgaggaagctgcagaatgggatagagtgcatccagtgcatgcagggcctattgcaccaggccagatgagagaaccaaggggaagtgacatagcaggaactactagtacccttcaggaacaaataggatggatgacacataatccacctatcccagtaggagaaatctataaaagatggataatcctgggattaaataaaatagtaagaatgtatagccctaccagcattctggacataagacaaggaccaaaggaaccctttagagactatgtagaccgattctataaaactctaagagccgagcaagcttcacaagaggtaaaaaattggatgacagaaaccttgttggtccaaaatgcgaacccagattgtaagactattttaaaagcattgggaccaggagcgacactagaagaaatgatgacagcatgtcagggagtggggggacccggccataaagcaagagttttggctgaagcaatgagccaagtaacaaatccagctaccataatgatacagaaaggcaattttaggaaccaaagaaagactgttaagtgtttcaattgtggcaaagaagggcacatagccaaaaattgcagggcccctaggaaaaagggctgttggaaatgtggaaaggaaggacaccaaatgaaagattgtactgagagacaggctaattttttagggaagatctggccttcccacaagggaaggccagggaattttcttcagagcagaccagagccaacagccccaccagaagagagcttcaggtttggggaagagacaacaactccctctcagaagcaggagccgatagacaaggaactgtatcctttagcttccctcagatcactctttggcagcgacccctcgtcacaataaagataggggggcaattaaaggaagctctattagatacaggagcagatgatacagtattagaagaaatgaatttgccaggaagatggaaaccaaaaatgatagggggaattggaggttttatcaaagtaagacagtatgatcagatactcatagaaatctgcggacataaagctataggtacagtattagtaggacctacacctgtcaacataattggaagaaatctgttgactcagattggctgcactttaaattttcccattagtcctattgagactgtaccagtaaaattaaagccaggaatggatggcccaaaagttaaacaatggccattgacagaagaaaaaataaaagcattagtagaaatttgtacagaaatggaaaaggaaggaaaaatttcaaaaattgggcctgaaaatccatacaatactccagtatttgccataaagaaaaaagacagtactaaatggagaaaattagtagatttcagagaacttaataagagaactcaagatttctgggaagttcaattaggaataccacatcctgcagggttaaaacagaaaaaatcagtaacagtactggatgtgggcgatgcatatttttcagttcccttagataaagacttcaggaagtatactgcatttaccatacctagtataaacaatgagacaccagggattagatatcagtacaatgtgcttccacagggatggaaaggatcaccagcaatattccagtgtagcatgacaaaaatcttagagccttttagaaaacaaaatccagacatagtcatctatcaatacatggatgatttgtatgtaggatctgacttagaaatagggcagcatagaacaaaaatagaggaactgagacaacatctgttgaggtggggatttaccacaccagacaaaaaacatcagaaagaacctccattcctttggatgggttatgaactccatcctgataaatggacagtacagcctatagtgctgccagaaaaggacagctggactgtcaatgacatacagaaattagtgggaaaattgaattgggcaagtcagatttatgcagggattaaagtaaggcaattatgtaaacttcttaggggaaccaaagcactaacagaagtagtaccactaacagaagaagcagagctagaactggcagaaaacagggagattctaaaagaaccggtacatggagtgtattatgacccatcaaaagacttaatagcagaaatacagaagcaggggcaaggccaatggacatatcaaatttatcaagagccatttaaaaatctgaaaacaggaaagtatgcaagaatgaagggtgcccacactaatgatgtgaaacaattaacagaggcagtacaaaaaatagccacagaaagcatagtaatatggggaaagactcctaaatttaaattacccatacaaaaggaaacatgggaagcatggtggacagagtattggcaagccacctggattcctgagtgggagtttgtcaatacccctcccttagtgaagttatggtaccagttagagaaagaacccataataggagcagaaactttctatgtagatggggcagccaatagggaaactaaattaggaaaagcaggatatgtaactgacagaggaagacaaaaagttgtccccctaacggacacaacaaatcagaagactgagttacaagcaattcatctagctttgcaggattcgggattagaagtaaacatagtgacagactcacaatatgcattgggaatcattcaagcacaaccagataagagtgaatcagagttagtcagtcaaataatagagcagttaataaaaaaggaaaaagtctacctggcatgggtaccagcacacaaaggaattggaggaaatgaacaagtagataaattggtcagtgctggaatcaggaaagtactatttttagatggaatagataaggcccaagaagaacatgagaaatatcacagtaattggagagcaatggctagtgattttaacctaccacctgtagtagcaaaagaaatagtagccagctgtgataaatgtcagctaaaaggggaagccatgcatggacaagtagactgtagcccaggaatatggcagctagattgtacacatttagaaggaaaagttatcttggtagcagttcatgtagccagtggatatatagaagcagaagtaattccagcagagacagggcaagaaacagcatacttcctcttaaaattagcaggaagatggccagtaaaaacagtacatacagacaatggcagcaatttcaccagtactacagttaaggccgcctgttggtgggcggggatcaagcaggaatttggcattccctacaatccccaaagtcaaggagtaatagaatctatgaataaagaattaaagaaaattataggacaggtaagagatcaggctgaacatcttaagacagcagtacaaatggcagtattcatccacaattttaaaagaaaaggggggattggggggtacagtgcaggggaaagaatagtagacataatagcaacagacatacaaactaaagaattacaaaaacaaattacaaaaattcaaaattttcgggtttattacagggacagcagagatccagtttggaaaggaccagcaaagctcctctggaaaggtgaaggggcagtagtaatacaagataatagtgacataaaagtagtgccaagaagaaaagcaaagatcatcagggattatggaaaacagatggcaggtgatgattgtgtggcaagtagacaggatgaggattaacacatggaattctgcaacaactgctgtttatccatttcagaattgggtgtcgacatagcagaataggcgttactcgacagaggagagcaagaaatggagccagtagatcctagactagagccctggaagcatccaggaagtcagcctaaaactgcttgtaccaattgctattgtaaaaagtgttgctttcattgccaagtttgtttcatgacaaaagccttaggcatctcctatggcaggaagaagcggagacagcgacgaagagctcatcagaacagtcagactcatcaagcttctctatcaaagcagtaagtagtacatgtaatgcaacctataatagtagcaatagtagcattagtagtagcaataataatagcaatagttgtgtggtccatagtaatcatagaatataggaaaatggccgctgatcttcagacctggaggaggagatatgagggacaattggagaagtgaattatataaatataaagtagtaaaaattgaaccattaggagtagcacccaccaaggcaaagagaagagtggtgcagagagaaaaaagagcagtgggaataggagctttgttccttgggttcttgggagcagcaggaagcactatgggcgcagcgtcaatgacgctgacggtacaggccagacaattattgtctggtatagtgcagcagcagaacaatttgctgagggctattgaggcgcaacagcatctgttgcaactcacagtctggggcatcaagcagctccaggcaagaatcctggctgtggaaagatacctaaaggatcaacagctcctggggatttggggttgctctggaaaactcatttgcaccactgctgtgccttggaatgctagttggagtaataaatctctggaacagatttggaatcacacgacctggatggagtgggacagagaaattaacaattacacaagcttaatacactccttaattgaagaatcgcaaaaccagcaagaaaagaatgaacaagaattattggaattagataaatgggcaagtttgtggaattggtttaacataacaaattggctgtggtatataaaattattcataatgatagtaggaggcttggtaggtttaagaatagtttttgctgtactttctatagtgaatagagttaggcagggatattcaccattatcgtttcagacccacctcccaaccccgaggggacccgacaggcccgaaggaatagaagaagaaggtggagagagagacagagacagatccattcgattagtgaacggatccttggcacttatctgggacgatctgcggagcctgtgcctcttcagctaccaccgcttgagagacttactcttgattgtaacgaggattgtggaacttctgggacgcagggggtgggaagccctcaaatattggtggaatctcctacaatattggagtcaggagctaaagaatagtgctgttagcttgctcaatgccacagccatagcagtagctgaggggacagatagggttatagaagtagtacaaggagcttgtagagctattcgccacatacctagaagaataagacagggcttggaaaggattttgctataagctcgaggccgccccggtgaccttcagaccttggcactggaggtggcccggcagaagcgcggcatcgtggatcagtgctgcaccagcatctgctctctctaccaactggagaactactgcaactaggcccaccactaccctgtccacccctctgcaatgaataaaacctttgaaagagcactacaagttgtgtgtacatgcgtgcatgtgcatatgtggtgcggggggaacatgagtggggctggctggagtggcgatgataagctgtcaaacatgagaattaattcttgaagacgaaagggcctcgtgatacgcctatttttataggttaatgtcatgataataatggtttcttagtctagaattaattccgtgtattctatagtgtcacctaaatcgtatgtgtatgatacataaggttatgtattaattgtagccgcgttctaacgacaatatgtacaagcctaattgtgtagcatctggcttactgaagcagaccctatcatctctctcgtaaactgccgtcagagtcggtttggttggacgaaccttctgagtttctggtaacgccgtcccgcacccggaaatggtcagcgaaccaatcagcagggtcatcgctagccagatcctctacgccggacgcatcgtggccggcatcaccggcgccacaggtgcggttgctggcgcctatatcgccgacatcaccgatggggaagatcgggctcgccacttcgggctcatgagcgcttgtttcggcgtgggtatggtggcaggccccgtggccgggggactgttgggcgccatctccttgcatgcaccattccttgcggcggcggtgctcaacggcctcaacctactactgggctgcttcctaatgcaggagtcgcataagggagagcgtcgaatggtgcactctcagtacaatctgctctgatgccgcatagttaagccagccccgacacccgccaacacccgctgacgcgccctgacgggcttgtctgctcccggcatccgcttacagacaagctgtgaccgtctccgggagctgcatgtgtcagaggttttcaccgtcatcaccgaaacgcgcgagacgaaagggcctcgtgatacgcctatttttataggttaatgtcatgataataatggtttcttagacgtcaggtggcacttttcggggaaatgtgcgcggaacccctatttgtttatttttctaaatacattcaaatatgtatccgctcatgagacaataaccctgataaatgcttcaataatattgaaaaaggaagagtatgagtattcaacatttccgtgtcgcccttattcccttttttgcggcattttgccttcctgtttttgctcacccagaaacgctggtgaaagtaaaagatgctgaagatcagttgggtgcacgagtgggttacatcgaactggatctcaacagcggtaagatccttgagagttttcgccccgaagaacgttttccaatgatgagcacttttaaagttctgctatgtggcgcggtattatcccgtattgacgccgggcaagagcaactcggtcgccgcatacactattctcagaatgacttggttgagtactcaccagtcacagaaaagcatcttacggatggcatgacagtaagagaattatgcagtgctgccataaccatgagtgataacactgcggccaacttacttctgacaacgatcggaggaccgaaggagctaaccgcttttttgcacaacatgggggatcatgtaactcgccttgatcgttgggaaccggagctgaatgaagccataccaaacgacgagcgtgacaccacgatgcctgtagcaatggcaacaacgttgcgcaaactattaactggcgaactacttactctagcttcccggcaacaattaatagactggatggaggcggataaagttgcaggaccacttctgcgctcggcccttccggctggctggtttattgctgataaatctggagccggtgagcgtgggtctcgcggtatcattgcagcactggggccagatggtaagccctcccgtatcgtagttatctacacgacggggagtcaggcaactatggatgaacgaaatagacagatcgctgagataggtgcctcactgattaagcattggtaactgtcagaccaagtttactcatatatactttagattgatttaaaacttcatttttaatttaaaaggatctaggtgaagatcctttttgataatctcatgaccaaaatcccttaacgtgagttttcgttccactgagcgtcagaccccgtagaaaagatcaaaggatcttcttgagatcctttttttctgcgcgtaatctgctgcttgcaaacaaaaaaaccaccgctaccagcggtggtttgtttgccggatcaagagctaccaactctttttccgaaggtaactggcttcagcagagcgcagataccaaatactgttcttctagtgtagccgtagttaggccaccacttcaagaactctgtagcaccgcctacatacctcgctctgctaatcctgttaccagtggctgctgccagtggcgataagtcgtgtcttaccgggttggactcaagacgatagttaccggataaggcgcagcggtcgggctgaacggggggttcgtgcacacagcccagcttggagcgaacgacctacaccgaactgagatacctacagcgtgagctatgagaaagcgccacgcttcccgaagggagaaaggcggacaggtatccggtaagcggcagggtcggaacaggagagcgcacgagggagcttccagggggaaacgcctggtatctttatagtcctgtcgggtttcgccacctctgacttgagcgtcgatttttgtgatgctcgtcaggggggcggagcctatggaaaaacgccagcaacgcggcctttttacggttcctggccttttgctggccttttgctcacatgttctttcctgcgttatcccctgattctgtggataaccgtattaccgcctttgagtgagctgataccgctcgccgcagccgaacgaccgagcgcagcgagtcagtgagcgaggaagcggaagagcgcccaatacgcaaaccgcctctccccgcgcgttggccgattcattaatgcagctgtggaatgtgtgtcagttagggtgtggaaagtccccaggctccccagcaggcagaagtatgcaaagcatgcatctcaattagtcagcaaccaggtgtggaaagtccccaggctccccagcaggcagaagtatgcaaagcatgcatctcaattagtcagcaaccatagtcccgcccctaactccgcccatcccgcccctaactccgcccagttccgcccattctccgccccatggctgactaattttttttatttatgcagaggccgaggccgcctcggcctctgagctattccagaagtagtgaggaggcttttttggaggcctaggcttttgcaaaaagcttggacacaagacaggcttgcgagatatgtttgagaataccactttatcccgcgtcagggagaggcagtgcgtaaaaagacgcggactcatgtgaaatactggtttttagtgcgccagatctctataatctcgcgcaacctattttcccctcgaacactttttaagccgtagataaacaggctgggacacttcacatgagcgaaaaatacatcgtcacctgggacatgttgcagatccatgcacgtaaactcgcaagccgactgatgccttctgaacaatggaaaggcattattgccgtaagccgtggcggtctgtaccgggtgcgttactggcgcgtgaactgggtattcgtcatgtcgataccgtttgtatttccagctacgatcacgacaaccagcgcgagcttaaagtgctgaaacgcgcagaaggcgatggcgaaggcttcatcgttattgatgacctggtggataccggtggtactgcggttgcgattcgtgaaatgtatccaaaagcgcactttgtcaccatcttcgcaaaaccggctggtcgtccgctggttgatgactatgttgttgatatcccgcaagatacctggattgaacagccgtgggatatgggcgtcgtattcgtcccgccaatctccggtcgctaatcttttcaacgcctggcactgccgggcgttgttctttttaacttcaggcgggttacaatagtttccagtaagtattctggaggctgcatccatgacacaggcaaacctgagcgaaaccctgttcaaaccccgctttaaacatcctgaaacctcgacgctagtccgccgctttaatcacggcgcacaaccgcctgtgcagtcggcccttgatggtaaaaccatccctcactggtatcgcatgattaaccgtctgatgtggatctggcgcggcattgacccacgcgaaatcctcgacgtccaggcacgtattgtgatgagcgatgccgaacgtaccgacgatgatttatacgatacggtgattggctaccgtggcggcaactggatttatgagtgggccccggatctttgtgaaggaaccttacttctgtggtgtgacataattggacaaactacctacagagatttaaagctctaaggtaaatataaaatttttaacccggatctttgtgaaggaaccttacttctgtggtgtgacataattggacaaactacctacagagatttaaagctctaaggtaaatataaaatttttaagtgtataatgtgttaaactactgattctaattgtttgtgtattttagattccaacctatggaactgatgaatgggagcagtggtggaatgcctttaatgaggaaaacctgttttgctcagaagaaatgccatctagtgatgatgaggctactgctgactctcaacattctactcctccaaaaaagaagagaaaggtagaagaccccaaggactttccttcagaattgctaagttttttgagtcatgctgtgtttagtaatagaactcttgcttgctttgctatttacaccacaaaggaaaaagctgcactgctatacaagaaaattatggaaaaatattctgtaacctttataagtaggcataacagttataatcataacatactgttttttcttactccacacaggcatagagtgtctgctattaataactatgctcaaaaattgtgtacctttagctttttaatttgtaaaggggttaataaggaatatttgatgtatagtgccttgactagagatcataatcagccataccacatttgtagaggttttacttgctttaaaaaacctcccacacctccccctgaacctgaaacataaaatgaatgcaattgttgttgttgggctgcaggaattaattcgagctcgcccgaca

SEQ ID NO: 2 - DNA, 16569 bp, synthetic construct
  source 1..16569: mol_type = other DNA; note = pXX6-80
cgggggtgcctcgacggggaaggtggtaggcgcgttggcggcatcggtggaggcggtggtggcgaactcagagggggcggttaggctgtccttcttctcgactgactccatgatctttttctgcctataggagaaggaaatggccagtcgggaagaggagcagcgcgaaaccacccccgagcgcggacgcggtgcggcgcgacgtcccccaaccatggaggacgtgtcgtccccgtccccgtcgccgccgcctccccgggcgcccccaaaaaagcggatgaggcggcgtatcgagtccgaggacgaggaagactcatcacaagacgcgctggtgccgcgcacacccagcccgcggccatcgacctcggcggcggatttggccattgcgcccaagaagaaaaagaagcgcccttctcccaagcccgagcgcccgccatcaccagaggtaatcgtggacagcgaggaagaaagagaagatgtggcgctacaaatggtgggtttcagcaacccaccggtgctaatcaagcatggcaaaggaggtaagcgcacagtgcggcggctgaatgaagacgacccagtggcgcgtggtatgcggacgcaagaggaagaggaagagcccagcgaagcggaaagtgaaattacggtgatgaacccgctgagtgtgccgatcgtgtctgcgtgggagaagggcatggaggctgcgcgcgcgctgatggacaagtaccacgtggataacgatctaaaggcgaacttcaaactactgcctgaccaagtggaagctctggcggccgtatgcaagacctggctgaacgaggagcaccgcgggttgcagctgaccttcaccagcaacaagacctttgtgacgatgatggggcgattcctgcaggcgtacctgcagtcgtttgcagaggtgacctacaagcatcacgagcccacgggctgcgcgttgtggctgcaccgctgcgctgagatcgaaggcgagcttaagtgtctacacggaagcattatgataaataaggagcacgtgattgaaatggatgtgacgagcgaaaacgggcagcgcgcgctgaaggagcagtctagcaaggccaagatcgtgaagaaccggtggggccgaaatgtggtgcagatctccaacaccgacgcaaggtgctgcgtgcacgacgcggcctgtccggccaatcagttttccggcaagtcttgcggcatgttcttctctgaaggcgcaaaggctcaggtggcttttaagcagatcaaggcttttatgcaggcgctgtatcctaacgcccagaccgggcacggtcaccttttgatgccactacggtgcgagtgcaactcaaagcctgggcacgcgccctttttgggaaggcagctaccaaagttgactccgttcgccctgagcaacgcggaggacctggacgcggatctgatctccgacaagagcgtgctggccagcgtgcaccacccggcgctgatagtgttccagtgctgcaaccctgtgtatcgcaactcgcgcgcgcagggcggaggccccaactgcgacttcaagatatcggcgcccgacctgctaaacgcgttggtgatggtgcgcagcctgtggagtgaaaacttcaccgagctgccgcggatggttgtgcctgagtttaagtggagcactaaacaccagtatcgcaacgtgtccctgccagtggcgcatagcgatgcgcggcagaacccctttgatttttaaacggcgcagacggcaagggtgggggtaaataatcacccgagagtgtacaaataaaagcatttgcctttattgaaagtgtctctagtacattatttttacatgtttttcaagtgacaaaaagaagtggcgctcctaatctgcgcactgtggctgcggaagtagggcgagtggcgctccaggaagctgtagagctgttcctggttgcgacgcagggtgggctgtacctggggactgttgagcatggagttgggtaccccggtaataaggttcatggtggggttgtgatccatgggagtttggggccagttggcaaaggcgtggagaaacatgcagcagaatagtccacaggcggccgagttgggcccctgtacgctttgggtggacttttccagcgttatacagcggtcgggggaagaagcaatggcgctacggcgcaggagtgactcgtactcaaactggtaaacctgcttgagtcgctggtcagaaaagccaaagggctcaaagaggtagcatgtttttgagtgcgggttccaggcaaaggccatccagtgtacgcccccagtctcgcgaccggccgtattgactatggcgcaggcgagcttgtgtggagaaacaaagcctggaaagcgcttgtcataggtgcccaaaaaatatggcccacaaccaagatctttgacaatggctttcagttcctgctcactggagcccatggcggcagctgttgttgatgttgcttgcttctttatgttgtggcgttgccggccgagaagggcgtgcgcaggtacacggtttcgatgacgccgcggtgcggctggtgcacacggaccacgtcaaagacttcaaacaaaacataaagaagggtgggctcgtccatgggatccacctcaaaagtcatgtctagcgcgtgggcggagttggcgtagagaaggttttggcccaggtctgtgagtgcgcccatggacataaagttactggagaatgggatgcgccaaagggtgcaaactgtgcaacgaggggatcttctgccgccggttggtcagcaggtagtttagggttgcctccaggctgcccgtgtcctcctgccccagcgcgcggctgacacttgtaatctcctggaaagtatgctcgtccacatgcgcctgacctatggcctcgcggtacagtgtcagcaagtgacctaggtatgtgtcccgggacacgctgccactgtccgtgaagggcgctattagcagcagcaacaggcgcgagttgggcgtcagcaagctagacacggtcgcgcggtcgcctgtgggagcccgcaccccccacagcccctgcaagtttttgaaagcctggctcaggtttacggtctgcaggccttgtctactggtctggaaaaaatagtctggcccagactggtacacctcactttgcggtgtctcagtcaccattagccgcagtgcgctcacaaagttggtgtagtcctcctgtccccgcggcacgttggcgggctgtgtactcaggaaggcgtttagtgcaaccatggagcccaggttgccctgctgctgcgcgcgctcacgctgcgccacggcctcgcgcacatcccccaccagccggtccaggttggtctgcacgttgccgctgttgtaacgagccacgcgctgaagcagcgcgtcgtagaccaggccggcctcgtcgggccggatggccctgttttcggccagcgcgtttacgatcgccagcaccttctcgtgcgtggggtttgcgcgcgccgggaccaccgcttccagaattgcggagagccggttggcctgcggctgctgccggaacgcgtcaggattgcgcgcagtcagcgacatgatgcggtccatgacctggcgccagtcgtccgtggagttaaggccggacggctggctctgcagcgccgcccgcaccgccgggtccgttgcgtcttgcatcatctgatcagaaacatcaccgcttagtactcgccgtcctctggctcgtactcatcgtcctcgtcatattcctccacgccgccgacgttgccagcgcgcgcgggtgccaccgccagcccaggtccggccccagctgcctccagggcgcgtcggcttggggcccagcgcaggtcagcgcccgcgtcaaagtaggactcggcctctctatcgccgctgcccgtgccagccagggccctttgcaggctgtgcatcagctcgcggtcgctgagctcgcgccgccggctcacgctcacggccttgtggatgcgctcgttgcgataaacgcccaggtcgtcgctcaaggtaagcaccttcagcgccatgcgcatgtagaacccctcgatctttacctccttgtctatgggaacgtaaggggtatggtatatcttgcgggcgtaaaacttgcccaggctaagcatggaatagttgatggcggccaccttgtcagccaggctcaagctgcgctcctgcaccactatgctctgcaggatgtttatcaaatcgagcagccagcggccctcgggctctactatgtttagcagcgcatccctgaatgcctcgttgtccctgctgtgctgcactataaggaacagctgcgccatgagcggcttgctatttgggttttgctccagcgcgcttacaaagtcccacagatgcatcagtcctatagccacctcctcgcgcgccacaagcgtacgcacgtggttgttaaagcttttttgaaagttaatctcctggttcaccgtctgctcgtatgcggttaccaggtcggcggccgccacgtgtgcgcgcgcgggactaatcccggttcgcgcgtcgggctcaaagtcctcctcgcgcagcaaccgctcgcgattcaggccatgccgcagctcgcgccctgcgtggaactttcgatcccgcatctcctcgggctcctctccctcgcggtcgcgaaacaggttctgccgcggcacgtacgcctcacgcgtatcacgcttcagctgcacccttgggtgccgctcaggagagggcgctcctagccgcgccaggccctcgccctcctccaagtccaggtagtgccgggcccggcgccgcgggggttcgtaatcaccatctgctgccgcgtcaaccgcggatgtcgcccctcctgacgcggtaggaggaggggagggtgccctgcatgtctgccgctgctcttgctcttgccgctgctgaggaggggggcgcatctgccgcagcaccggatgcatctgggaaaagcaaaaaaggggctcgtccctgtttccggaggaatttgcaagcggggtcttgcatgacggggaggcaaacccccgttcgccgcagtccggccggtccgagactcgaaccgggggtcccgcgactcaacccttggaaaataaccctccggctacagggagcgagccacttaatgctttcgctttccagcctaaccgcttacgctgcgcgcggccagtggccaaaaaagctagcgcagcagccgccgcgcctggaaggaagccaaaaggagcactcccccgttgtctgacgtcgcacacctgggttcgacacgcgggcggtaaccgcatggatcacggcggacggccggatacggggctcgaaccccggtcgtccgccatgatacccttgcgaatttatccaccagaccacggaagagtgcccgcttacaggctctccttttgcacgctagagcgtcaacgattgcgcgcgcctgaccggccagagcgtcccgaccatggagcactttttgccgctgcgcaacatctggaaccgcgtccgcgactttccgcgcgcctccaccaccgccgccggcatcacctggatgtccaggtacatctacggatatcatcgccttatgttggaagatctcgcccccggagccccggccaccctacgctggcccctctaccgccagccgccgccgcactttttggtgggataccagtacctggtgcggacttgcaacgactacgtatttgactcgagggcttactcgcgtctcaggtacaccgagctctcgcagccgggtcaccagaccgttaactggtccgttatggccaactgcacttacaccatcaacacgggcgcataccaccgctttgtggacatggatgacttccagtctaccctcacgcaggtgcagcaggccatattagccgagcgcgttgtcgccgacctagccctgcttcagccgatgaggggcttcggggtcacacgcatgggaggaagagggcgccacctacggccaaactccgccgccgccgcagcgatagatgcaagagatgcaggacaagaggaaggagaagaagaagtgccggtagaaaggctcatgcaagactactacaaagacctgcgccgatgtcaaaacgaagcctggggcatggccgaccgcctgcgcattcagcaggccggacccaaggacatggtgcttctgtcgagaagtactagtggccacgtgggccgtgcaccttaagcttggcactggccgtcgttttacaacgtcgtgactgggaaaaccctggcgttacccaacttaatcgccttgcagcacatccccctttcgccagctggcgtaatagcgaagaggcccgcaccgatcgcccttcccaacagttgcgcagcctgaatggcgaatggcgcctgatgcggtattttctccttacgcatctgtgcggtatttcacaccgcatacgtcaaagcaaccatagtacgcgccctgtagcggcgcattaagcgcggcgggtgtggtggttacgcgcagcgtgaccgctacacttgccagcgccctagcgcccgctcctttcgctttcttcccttcctttctcgccacgttcgccggctttccccgtcaagctctaaatcgggggctccctttagggttccgatttagtgctttacggcacctcgaccccaaaaaacttgatttgggtgatggttcacgtagtgggccatcgccctgatagacggtttttcgccctttgacgttggagtccacgttctttaatagtggactcttgttccaaactggaacaacactcaaccctatctcgggctattcttttgatttataagggattttgccgatttcggcctattggttaaaaaatgagctgatttaacaaaaatttaacgcgaattttaacaaaatattaacgtttacaattttatggtgcactctcagtacaatctgctctgatgccgcatagttaagccagccccgacacccgccaacacccgctgacgcgccctgacgggcttgtctgctcccggcatccgcttacagacaagctgtgaccgtctccgggagctgcatgtgtcagaggttttcaccgtcatcaccgaaacgcgcgagacgaaagggcctcgtgatacgcctatttttataggttaatgtcatgataataatggtttcttagacgtcaggtggcacttttcggggaaatgtgcgcggaacccctatttgtttatttttctaaatacattcaaatatgtatccgctcatgagacaataaccctgataaatgcttcaataatattgaaaaaggaagagtatgagtattcaacatttccgtgtcgcccttattcccttttttgcggcattttgccttcctgtttttgctcacccagaaacgctggtgaaagtaaaagatgctgaagatcagttgggtgcacgagtgggttacatcgaactggatctcaacagcggtaagatccttgagagttttcgccccgaagaacgttttccaatgatgagcacttttaaagttctgctatgtggcgcggtattatcccgtattgacgccgggcaagagcaactcggtcgccgcatacactattctcagaatgacttggttgagtactcaccagtcacagaaaagcatcttacggatggcatgacagtaagagaattatgcagtgctgccataaccatgagtgataacactgcggccaacttacttctgacaacgatcggaggaccgaaggagctaaccgcttttttgcacaacatgggggatcatgtaactcgccttgatcgttgggaaccggagctgaatgaagccataccaaacgacgagcgtgacaccacgatgcctgtagcaatggcaacaacgttgcgcaaactattaactggcgaactacttactctagcttcccggcaacaattaatagactggatggaggcggataaagttgcaggaccacttctgcgctcggcccttccggctggctggtttattgctgataaatctggagccggtgagcgtgggtctcgcggtatcattgcagcactggggccagatggtaagccctcccgtatcgtagttatctacacgacggggagtcaggcaactatggatgaacgaaatagacagatcgctgagataggtgcctcactgattaagcattggtaactgtcagaccaagtttactcatatatactttagattgatttaaaacttcatttttaatttaaaaggatctaggtgaagatcctttttgataatctcatgaccaaaatcccttaacgtgagttttcgttccactgagcgtcagaccccgtagaaaagatcaaaggatcttcttgagatcctttttttctgcgcgtaatctgctgcttgcaaacaaaaaaaccaccgctaccagcggtggtttgtttgccggatcaagagctaccaactctttttccgaaggtaactggcttcagcagagcgcagataccaaatactgttcttctagtgtagccgtagttaggccaccacttcaagaactctgtagcaccgcctacatacctcgctctgctaatcctgttaccagtggctgctgccagtggcgataagtcgtgtcttaccgggttggactcaagacgatagttaccggataaggcgcagcggtcgggctgaacggggggttcgtgcacacagcccagcttggagcgaacgacctacaccgaactgagatacctacagcgtgagctatgagaaagcgccacgcttcccgaagggagaaaggcggacaggtatccggtaagcggcagggtcggaacaggagagcgcacgagggagcttccagggggaaacgcctggtatctttatagtcctgtcgggtttcgccacctctgacttgagcgtcgatttttgtgatgctcgtcaggggggcggagcctatggaaaaacgccagcaacgcggcctttttacggttcctggccttttgctggccttttgctcacatgttctttcctgcgttatcccctgattctgtggataaccgtattaccgcctttgagtgagctgataccgctcgccgcagccgaacgaccgagcgcagcgagtcagtgagcgaggaagcggaagagcgcccaatacgcaaaccgcctctccccgcgcgttggccgattcattaatgcagctggcacgacaggtttcccgactggaaagcgggcagtgagcgcaacgcaattaatgtgagttagctcactcattaggcaccccaggctttacactttatgcttccggctcgtatgttgtgtggaattgtgagcggataacaatttcacacaggaaacagctatgacatgattacgaattcgataagctttaatgcggtagtttatcacagttaaattgctaacgcagtcaggcaccgtgtatgaaatctaacaatgcgctcatcgtcatcctcggcaccgtcaccctggatgctgtaggcataggcttggttatgccggtactgccgggcctcttgcgggatatcgtccattccgacagcatcgccagtcactatggcgtgctgctagcgctatatgcgttgatgcaatttctatgcgcacccgttctcggagcactgtccgaccgctttggccgccgcccagtcctgctcgcttcgctacttggagccactatcgactacgcgatcatggcgaccacacccgtcctgtggatccggcgcacaccaaaaacgtcacttttgccacatccgtcgcttacatgtgttccgccacacttgcaacatcacacttccgccacactactacgtcacccgccccgttcccacgccccgcgccacgtcacaaactccaccccctcattatcatattggcttcaatccaaaataaggtatattattgatgattattttggattgaagccaatatgataatgagggggtggagtttgtgacgtgggggggcgtgggaacggggcgggtgacgtaggttttagggcggagtaacttgtatgtgttgggaattgtagttttcttaaaatgggaagtgacgtaacgtgggaaaacggaagtgacgatttgaggaagttgtgggttttttggctttcgtttctgggcgtaggttcgcgtgcggttttctgggtgttttttgtggactttaaccgttacgtcattttttagtcctatatatactcgctctgcacttggcccttttttacactgtgactgattgagctggtgccgtgtcgagtggtgtttttttaataggttttcttttttactggtaaggctgactgttatggctgccgctgtggaagcgctgtatgttgttctggagcgggagggtgctattttgcctaggcaggagggtttttcaggtgtttatgtgtttttctctcctattaattttgttatacctcctatgggggctgtaatgttgtctctacgcctgcgggtatgtattcccccgggctatttcggtcgctttttagcactgaccgatgtgaatcaacctgatgtgtttaccgagtcttacattatgactccggacatgaccgaggagctgtcggtggtgctttttaatcacggtgaccagtttttttacggtcacgccggcatggccgtagtccgtcttatgcttataagggttgtttttcctgttgtaagacaggcttctaatgtttaaatgtttttttgttattttattttgtgtttatgcagaaacccgcagacatgtttgagagaaaaatggtgtctttttctgtggtggttccggagcttacctgcctttatctgcatgagcatgactacgatgtgctttcttttttgcgcgaggctttgcctgattttttgagcagcaccttgcattttatatcgccgcccatgcaacaagcttacatcggggctacgctggttagcatagctccgagtatgcgtgtcataatcagtgtgggttcttttgtcatggttcctggcggggaagtggccgcgctggtccgtgcagacctgcacgattatgttcagctggccctgcgaagggacctacgggatcgcggtatttttgttaatgttccgcttttgaatcttatacaggtctgtgaggaacctgaatttttgcaatcatgattcgctgcttgaggctgaaggtggagggcgctctggagcagatttttacaatggccggacttaatattcgggatttgcttagagatatattgagaaggtggcgagatgagaattatttgggcatggttgaaggtgctggaatgtttatagaggagattcaccctgaagggtttagcctttacgtccacttggacgtgagggccgtttgccttttggaagccattgtgcaacatcttacaaatgccattatctgttctttggctgtagagtttgaccacgccaccggaggggagcgcgttcacttaatagatcttcattttgaggttttggataatcttttggaataaaaaaaaaaacatggttcttccagctcttcccgctcctcccgtgtgtgactcgcagaacgaatgtgtaggttggctgggtgtggcttattctgcggtggtggatgttatcagggcagcggcgcatgaaggagtttacatagaacccgaagccagggggcgcctggatgctttgagagagtggatatactacaactactacacagagcgatctaagcggcgagaccggagacgcagatctgtttgtcacgcccgcacctggttttgcttcaggaaatatgactacgtccggcgttccatttggcatgacactacgaccaacacgatctcggttgtctcggcgcactccgtacagtagggatcgtctacctccttttgagacagaaacccgcgctaccatactggaggatcatccgctgctgcccgaatgtaacactttgacaatgcacaacgtgagttacgtgcgaggtcttccctgcagtgtgggatttacgctgattcaggaatgggttgttccctgggatatggttctaacgcgggaggagcttgtaatcctgaggaagtgtatgcacgtgtgcctgtgttgtgccaacattgatatcatgacgagcatgatgatccatggttacgagtcctgggctctccactgtcattgttccagtcccggttccctgcagtgtatagccggcgggcaggttttggccagctggtttaggatggtggtggatggcgccatgtttaatcagaggtttatatggtaccgggaggtggtgaattacaacatgccaaaagaggtaatgtttatgtccagcgtgtttatgaggggtcgccacttaatctacctgcgcttgtggtatgatggccacgtgggttctgtggtccccgccatgagctttggatacagcgccttgcactgtgggattttgaacaatattgtggtgctgtgctgcagttactgtgctgatttaagtgagatcagggtgcgctgctgtgcccggaggacaaggcgccttatgctgcgggcggtgcgaatcatcgctgaggagaccactgccatgttgtattcctgcaggacggagcggcggcggcagcagtttattcgcgcgctgctgcagcaccaccgccctatcctgatgcacgattatgactctacccccatgtaggcgtggacttctccttcgccgcccgttaagcaaccgcaagttggacagcagcctgtggctcagcagctggacagcgacatgaacttaagtgagctgcccggggagtttattaatatcactgatgagcgtttggctcgacaggaaaccgtgtggaatataacacctaagaatatgtctgttacccatgatatgatgctttttaaggccagccggggagaaaggactgtgtactctgtgtgttgggagggaggtggcaggttgaatactagggttctgtgagtttgattaaggtacggtgatctgtataagctatgtggtggtggggctatactactgaatgaaaaatgacttgaaattttctgcaattgaaaaataaacacgttgaaacataacacaaacgattctttattcttgggcaatgtatgaaaaagtgtaagaggatgtggcaaatatttcattaatgtagttgtggccagaccagtcccatgaaaatgacatagagtatgcacttggagttgtgtctcctgtttcctgtgtaccgtttagtgtaatggttagtgttacaggtttagttttgtctccgtttaagtaaacttgactgacaatgttacttttggcagttttaccgtgagattttggataagctgataggttaggcataaatccaacagcgtttgtataggctgtgccttcagtaagatctccatttctaaagttccaatattctgggtccaggaaggaattgtttagtagcactccattttcgtcaaatcttataataagatgagcactttgaactgttccagatattggagccaaactgcctttaacagccaaaactgaaactgtagcaagtatttgactgccacattttgttaagaccaaagtgagtttagcatctttctctgcatttagtctacagttaggagatggagctggtgtggtccacaaagttagcttatcattatttttgtttcctactgtaatggcacctgtgctgtcaaaactaaggccagttcctagtttaggaaccatagccttgtttgaatcaaattctaggccatggccaatttttgttttgaggggatttgtgtttggtgcattaggtgaaccaaattcaagcccatctcctgcattaatggctatggctgtagcgtcaaacatcaaccccttggcagtgcttaggttaacctcaagctttttggaattgtttgaagctgtaaacaagtaaaggcctttgttgtagttaatatccaagttgtgggctgagtttataaaaagagggccctgtcctagtcttagatttagttggttttgagcatcaaacggataactaacatcaagtataaggcgtctgttttgagaatcaatccttagtcctcctgctacattaagttgcatattgccttgtgaatcaaaacccaaggctccagtaactttagtttgcaaggaagtattattaatagtcacacctggaccagttgctacggtcaaagtgtttaggtcgtctgttacatgcaaaggagccccgtactttagtcctagttttccattttgtgtataaatgggctctttcaagtcaatgcccaagctaccagtggcagtagttagagggggtgaggcagtgatagtaagggtactgctatcggtggtggtgagggggcctgatgtttgcagggctagctttccttctgacactgtgaggggtccttgggtggcaatgctaagtttggagtcgtgcacggttagcggggcctgtgattgcatggtgagtgtgttgcccgcgaccattagaggtgcggcggcagccacagttagggcttctgaggtaactgtgaggggtgcagatatttccaggtttatgtttgacttggtttttttgagaggtgggctcacagtggttacattttgggaggtaaggttgccggcctcgtccagagagaggccgttgcccattttgagcgcaagcatgccattggaggtaactagaggttcggataggcgcaaagagagtaccccagggggactctcttgaaacccattgggggatacaaagggaggagtaagaaaaggcacagttggaggaccggtttccgtgtcatatggatacacggggttgaaggtatcttcagacggtcttgcgcgcttcatctgcaacaacatgaagatagtgggtgcggatggacaggaacaggaggaaactgacattccatttagattgtggagaaagtttgcagccaggaggaagctgcaataccagagctgggaggagggcaaggaggtgctgctgaataaactggacagaaatttgctaactgattttaagtaagtgatgctttattatttttttttattagttaaagggaataagatccccgggtactctagttaattaactagaggatcttgatgtaatccagggttaggacagttgcaaatcacagtgagaacacagggtcccctgtcccgctcaactagcagggggcgctgggtaaactcccgaatcaggctacgggcaagctctccctgggcggtaagccggacgccgtgcgccgggccctcgatatgatcctcgggcaattcaaagtagcaaaactcaccggagtcgcgggcaaagcacttgtggcggcgacagtggaccaggtgtttcaggcgcagttgctctgcctctccacttaacattcagtcgtagccgtccgccgagtcctttaccgcgtcaaagttaggaataaattgatccggatagtggccgggaggtcccgagaaggggttaaagtagaccgatggcacaaactcctcaataaattgcagagttccaatgcctccagagcgcggctcagaggacgaggtctgcagagttaggattgcctgacgaggcgtgaatgaagagcggccggcgccgccgatctgaaatgtcccgtccggacggagaccaagcgaggagctcaccgactcgtcgttgagctgaatacctcgccctctgattgtcaggtgagttataccctgcccgggcgaccgcaccctgtgacgaaagccgcccgcaagctgcgcccctgagttagtcatctgaacttcggcctgggcgtctctgggaagtaccacagtggtgggagcgggactttcctggtacaccagggcagcgggccaactacggggattaaggttattacgaggtgtggtggtaatagccgcctgttccaggagaattcggtttcggtgggcgcgtattccgttgacccgggatatcatgtggggtcccgcgctcatgtagtttattcgggttgagtagtcttgggcagctccagccgcaagtcccatttgtggctggtaactccacatgtagggcgtgggaatttccttgctcataatggcgctgacaacaggtgctggcgccgggtgtggccgctggagatgacgtagttttcgcgcttaaatttgagaaagggcgcgaaactagtccttaagagtcagcgcgcagtatttactgaagagagcctccgcgtcttccagcgtgcgccgaagctgatcttcgcttttgtgatacaggcagctgcgggtgagggatcgcagagacctgttttttattttcagctcttgttcttggcccctgctctgttgaaatatagcatacagagtgggaaaaatcctgtttctaagctcgcgggtcgatacgggttcgttgggcgccagacgcagcgctcctcctcctgctgctgccgccgctgtggatttcttgggctttgtcagagtcttgctatccggtcgcctttgcttctgtgtggccgctgctgttgctgccgctgccgccggtgcagtatgggctgtagagatgacggtagtaatgcaggatgttacgggggaaggccacgccgtgatggtagagaagaaagcggcgggcgaaggagatgttgcccccacagtcttgcaagcaagcaactatggcgttcttgtgcccgcgccatgagcggtagccttggcgctgttgttgctcttgggctaacggcggcgg

SEQ ID NO: 3 - DNA, 5333 bp, synthetic construct
  source 1..5333: mol_type = other DNA; note = pscAAV-SFFV-eGFP
ggttcctggccttttgctggccttttgctcacatgttctttcctgcgttatcccctgattctgtggataaccgtattaccgcctttgagtgagctgataccgctcgccgcagccgaacgaccgagcgcagcgagtcagtgagcgaggaagcggaagagcgcccaatacgcaaaccgcctctccccgcgcgttggccgattcattaatgcagctggcgcgctcgctcgctcactgaggccgcccgggcaaagcccgggcgtcgggcgacctttggtcgcccggcctcagtgagcgagcgagcgcgcagagagggagtgggtcgttctagtcgaccaattctcataatgaaagaccccacctgtaggtttggcaagctagctgcagtaacgccattttgcaaggcatggaaaaataccaaaccaagaatagagaagttcagatcaagggcgggtacatgaaaatagctaacgttgggccaaacaggatatctgcggtgagcagtttcggccccggcccggggccaagaacagatggtcaccgcagtttcggccccggcccgaggccaagaacagatggtccccagatatggcccaaccctcagcagtttcttaagacccatcagatgtttccaggctcccccaaggacctgaaatgaccctgcgccttatttgaattaaccaatcagcctgcttctcgcttctgttcgcgcgcttctgcttcccgagctctataaaagagctcacaacccctcactcggcgcgccagtcctccgacagactgagtcgcccggggctgggtaccgcgggcccgggatccatcgccaccatggtgagcaagggcgaggagctgttcaccggggtggtgcccatcctggtcgagctggacggcgacgtaaacggccacaagttcagcgtgtccggcgagggcgagggcgatgccacctacggcaagctgaccctgaagttcatctgcaccaccggcaagctgcccgtgccctggcccaccctcgtgaccaccctgacctacggcgtgcagtgcttcagccgctaccccgaccacatgaagcagcacgacttcttcaagtccgccatgcccgaaggctacgtccaggagcgcaccatcttcttcaaggacgacggcaactacaagacccgcgccgaggtgaagttcgagggcgacaccctggtgaaccgcatcgagctgaagggcatcgacttcaaggaggacggcaacatcctggggcacaagctggagtacaactacaacagccacaacgtctatatcatggccgacaagcagaagaacggcatcaaggtgaacttcaagatccgccacaacatcgaggacggcagcgtgcagctcgccgaccactaccagcagaacacccccatcggcgacggccccgtgctgctgcccgacaaccactacctgagcacccagtccgccctgagcaaagaccccaacgagaagcgcgatcacatggtcctgctggagttcgtgaccgccgccgggatcactctcggcatggacgagctgtacaagtaaagcggccgccctgcaggctcgactgtgccttctagttgccagccatctgttgtttgcccctcccccgtgccttccttgaccctggaaggtgccactcccactgtcctttcctaataaaatgaggaaattgcatcgcattgtctgagtaggtgtcattctattctggggggtggggtggggcaggacagcaagggggaggattgggaagacaatagcaggcatgctggggatgcggtgggctctatggctcgagcatggcgggttaatcattaactacaaggaacccctagtgatggagttggccactccctctctgcgcgctcgctcgctcactgaggccgggcgaccaaaggtcgcccgacgcccgggctttgcccgggcggcctcagtgagcgagcgagcgcgcagctggcgtaatagcgaagaggcccgcaccgatcgcccttcccaacagttgcgcagcctgaatggcgaatggcgattccgttgcaatggctggcggtaatattgttctggatattaccagcaaggccgatagtttgagttcttctactcaggcaagtgatgttattactaatcaaagaagtattgcgacaacggttaatttgcgtgatggacagactcttttactcggtggcctcactgattataaaaacacttctcaggattctggcgtaccgttcctgtctaaaatccctttaatcggcctcctgtttagctcccgctctgattctaacgaggaaagcacgttatacgtgctcgtcaaagcaaccatagtacgcgccctgtagcggcgcattaagcgcggcgggtgtggtggttacgcgcagcgtgaccgctacacttgccagcgccctagcgcccgctcctttcgctttcttcccttcctttctcgccacgttcgccggctttccccgtcaagctctaaatcgggggctccctttagggttccgatttagtgctttacggcacctcgaccccaaaaaacttgattagggtgatggttcacgtagtgggccatcgccctgatagacggtttttcgccctttgacgttggagtccacgttctttaatagtggactcttgttccaaactggaacaacactcaaccctatctcggtctattcttttgatttataagggattttgccgatttcggcctattggttaaaaaatgagctgatttaacaaaaatttaacgcgaattttaacaaaatattaacgtttacaatttaaatatttgcttatacaatcttcctgtttttggggcttttctgattatcaaccggggtacatatgattgacatgctagttttacgattaccgttcatcgattctcttgtttgctccagactctcaggcaatgacctgatagcctttgtagagacctctcaaaaatagctaccctctccggcatgaatttatcagctagaacggttgaatatcatattgatggtgatttgactgtctccggcctttctcacccgtttgaatctttacctacacattactcaggcattgcatttaaaatatatgagggttctaaaaatttttatccttgcgttgaaataaaggcttctcccgcaaaagtattacagggtcataatgtttttggtacaaccgatttagctttatgctctgaggctttattgcttaattttgctaattctttgccttgcctgtatgatttattggatgttggaanttcctgatgcggtattttctccttacgcatctgtgcggtatttcacaccgcatatggtgcactctcagtacaatctgctctgatgccgcatagttaagccagccccgacacccgccaacacccgctgacgcgccctgacgggcttgtctgctcccggcatccgcttacagacaagctgtgaccgtctccgggagctgcatgtgtcagaggttttcaccgtcatcaccgaaacgcgcgagacgaaagggcctcgtgatacgcctatttttataggttaatgtcatgataataatggtttcttagacgtcaggtggcacttttcggggaaatgtgcgcggaacccctatttgtttatttttctaaatacattcaaatatgtatccgctcatgagacaataaccctgataaatgcttcaataatattgaaaaaggaagagtatgagtattcaacatttccgtgtcgcccttattcccttttttgcggcattttgccttcctgtttttgctcacccagaaacgctggtgaaagtaaaagatgctgaagatcagttgggtgcacgagtgggttacatcgaactggatctcaacagcggtaagatccttgagagttttcgccccgaagaacgttttccaatgatgagcacttttaaagttctgctatgtggcgcggtattatcccgtattgacgccgggcaagagcaactcggtcgccgcatacactattctcagaatgacttggttgagtactcaccagtcacagaaaagcatcttacggatggcatgacagtaagagaattatgcagtgctgccataaccatgagtgataacactgcggccaacttacttctgacaacgatcggaggaccgaaggagctaaccgcttttttgcacaacatgggggatcatgtaactcgccttgatcgttgggaaccggagctgaatgaagccataccaaacgacgagcgtgacaccacgatgcctgtagcaatggcaacaacgttgcgcaaactattaactggcgaactacttactctagcttcccggcaacaattaatagactggatggaggcggataaagttgcaggaccacttctgcgctcggcccttccggctggctggtttattgctgataaatctggagccggtgagcgtgggtctcgcggtatcattgcagcactggggccagatggtaagccctcccgtatcgtagttatctacacgacggggagtcaggcaactatggatgaacgaaatagacagatcgctgagataggtgcctcactgattaagcattggtaactgtcagaccaagtttactcatatatactttagattgatttaaaacttcatttttaatttaaaaggatctaggtgaagatcctttttgataatctcatgaccaaaatcccttaacgtgagttttcgttccactgagcgtcagaccccgtagaaaagatcaaaggatcttcttgagatcctttttttctgcgcgtaatctgctgcttgcaaacaaaaaaaccaccgctaccagcggtggtttgtttgccggatcaagagctaccaactctttttccgaaggtaactggcttcagcagagcgcagataccaaatactgtccttctagtgtagccgtagttaggccaccacttcaagaactctgtagcaccgcctacatacctcgctctgctaatcctgttaccagtggctgctgccagtggcgataagtcgtgtcttaccgggttggactcaagacgatagttaccggataaggcgcagcggtcgggctgaacggggggttcgtgcacacagcccagcttggagcgaacgacctacaccgaactgagatacctacagcgtgagctatgagaaagcgccacgcttcccgaagggagaaaggcggacaggtatccggtaagcggcagggtcggaacaggagagcgcacgagggagcttccagggggaaacgcctggtatctttatagtcctgtcgggtttcgccacctctgacttgagcgtcgatttttgtgatgctcgtcaggggggcggagcctatggaaaaacgccagcaacgcggcctttttac

SEQ ID NO: 4 - DNA, 7398 bp, synthetic construct
  source 1..7398: mol_type = other DNA; note = pRC26 AAV6wt
gggatccgctcgttctagagtcctgtattagaggtcacgtgagtgttttgcgacattttgcgacaccatgtggtcacgctgggtatttaagcccgagtgagcacgcagggtctccattttgaagcgggaggtttgaacgcgcagccgccatgccggggttttacgagattgtgattaaggtccccagcgaccttgacgagcatctgcccggcatttctgacagctttgtgaactgggtggccgagaaggaatgggagttgccgccagattctgacatggatctgaatctgattgagcaggcacccctgaccgtggccgagaagctgcagcgcgactttctgacggaatggcgtcgtgtgagtaaggccccggaagcccttttctttgtgcaatttgagaagggagagagctacttccacatgcacgtgctcgtggaaaccaccggggtgaaatctatggttttgggacgtttcctgagtcagattcgcgaaaaactgattcagagaatttaccgcgggatcgagccgactttgccaaactggttcgcggtcacaaagaccagaaatggtgccggaggcgggaacaaggtggtggatgagtgctacatccccaattacttgctccccaaaacccagcctgagctccagtgggcgtggactaatatggaacagtatttaagcgcctgtttgaatctcacggagcgtaaacggttggtggcgcagcatctgacgcacgtgtcgcagacgcaggagcagaacaaagagaatcagaatcccaattctgatgcgccggtgatcagatcaaaaacttcagccaggtacatggagctggtcgggtggctcgtggacaaggggattacctcggagaagcagtggatacaggaggaccaggcctcatacatctccttcaatgcggcctccaactcgcggtcccaaatcaaggctgccttggacaatgcgggaaagattatgagcctgactaaaaccgcccccgactacctggtgggccagcagcccgtggaggacatttccagcaatcggatttataaaattttggaactaaacgggtacgatccccaatatgcggcttccgtctttctgggatgggccacgaaaaagttcggcaagaggaacaccatctggctgtttgggcctgcaactaccgggaagaccaacatcgcggaggccatagcccacactgtgcccttctacgggtgcgtaaactggaccaatgagaactttcccttcaacgactgtgtcgacaagatggtgatctggtgggaggaggggaagatgaccgccaaggtcgtggagtcggccaaagccattctcggaggaagcaaggtgcgcgtggaccagaaatgcaagtcctcggcccagatagacccgactcccgtgatcgtcacctccaacaccaacatgtgcgccgtgattgacgggaactcaacgaccttcgaacaccagcagccgttgcaagaccggatgttcaaatttgaactcacccgccgtctggatcatgactttgggaaggtcaccaagcaggaagtcaaagactttttccggtgggcaaaggatcacgtggttgaggtggagcatgaattctacgtcaaaaagggtggagccaagaaaagacccgcccccagtgacgcagatataagtgagcccaaacgggtgcgcgagtcagttgcgcagccatcgacgtcagacgcggaagcttcgatcaactacgcagacaggtaccaaaacaaatgttctcgtcacgtgggcatgaatctgatgctgtttccctgcagacaatgcgagagaatgaatcagaattcaaatatctgcttcactcacggacagaaagactgtttagagtgctttcccgtgtcagaatctcaacccgtttctgtcgtcaaaaaggcgtatcagaaactgtgctacattcatcatatcatgggaaaggtgccagacgcttgcactgcctgcgatctggtcaatgtggatttggatgactgcatctttgaacaataaatgatttaaatcaggtatggctgccgatggttatcttccagattggctcgaggacaacctctctgagggcattcgcgagtggtgggacttgaaacctggagccccgaaacccaaagccaaccagcaaaagcaggacgacggccggggtctggtgcttcctggctacaagtacctcggacccttcaacggactcgacaagggggagcccgtcaacgcggcggatgcagcggccctcgagcacgacaaggcctacgaccagcagctcaaagcgggtgacaatccgtacctgcggtataaccacgccgacgccgagtttcaggagcgtctgcaagaagatacgtcttttgggggcaacctcgggcgagcagtcttccaggccaagaagagggttctcgaaccttttggtctggttgaggaaggtgctaagacggctcctggaaagaaacgtccggtagagcagtcgccacaagagccagactcctcctcgggcattggcaagacaggccagcagcccgctaaaaagagactcaattttggtcagactggcgactcagagtcagtccccgacccacaacctctcggagaacctccagcaacccccgctgctgtgggacctactacaatggcttcaggcggtggcgcaccaatggcagacaataacgaaggcgccgacggagtgggtaatgcctcaggaaattggcattgcgattccacatggctgggcgacagagtcatcaccaccagcacccgaacatgggccttgcccacctataacaaccacctctacaagcaaatctccagtgcttcaacgggggccagcaacgacaaccactacttcggctacagcaccccctgggggtattttgatttcaacagattccactgccatttctcaccacgtgactggcagcgactcatcaacaacaattggggattccggcccaagagactcaacttcaagctcttcaacatccaagtcaaggaggtcacgacgaatgatggcgtcacgaccatcgctaataaccttaccagcacggttcaagtcttctcggactcggagtaccagttgccgtacgtcctcggctctgcgcaccagggctgcctccctccgttcccggcggacgtgttcatgattccgcagtacggctacctaacgctcaacaatggcagccaggcagtgggacggtcatccttttactgcctggaatatttcccatcgcagatgctgagaacgggcaataactttaccttcagctacaccttcgaggacgtgcctttccacagcagctacgcgcacagccagagcctggaccggctgatgaatcctctcatcgaccagtacctgtattacctgaacagaactcagaatcagtccggaagtgcccaaaacaaggacttgctgtttagccgggggtctccagctggcatgtctgttcagcccaaaaactggctacctggaccctgttaccggcagcagcgcgtttctaaaacaaaaacagacaacaacaacagcaactttacctggactggtgcttcaaaatataaccttaatgggcgtgaatctataatcaaccctggcactgctatggcctcacacaaagacgacaaagacaagttctttcccatgagcggtgtcatgatttttggaaaggagagcgccggagcttcaaacactgcattggacaatgtcatgatcacagacgaagaggaaatcaaagccactaaccccgtggccaccgaaagatttgggactgtggcagtcaatctccagagcagcagcacagaccctgcgaccggagatgtgcatgttatgggagccttacctggaatggtgtggcaagacagagacgtatacctgcagggtcctatttgggccaaaattcctcacacggatggacactttcacccgtctcctctcatgggcggctttggacttaagcacccgcctcctcagatcctcatcaaaaacacgcctgttcctgcgaatcctccggcagagttttcggctacaaagtttgcttcattcatcacccagtattccacaggacaagtgagcgtggagattgaatgggagctgcagaaagaaaacagcaaacgctggaatcccgaagtgcagtatacatctaactatgcaaaatctgccaacgttgatttcactgtggacaacaatggactttatactgagcctcgccccattggcacccgttacctcacccgtcccctgtaattggcaggtcttgttaatcaataaaccgtttaattcgtttcagttgaactttggtccctgcgtatttctttcttatctagtttccatgctctagagcggccgccaccgcggtggagctccagcttttgttccctttagtgagggttaattgcgcgcttggcgtaatcatggtcatagctgtttcctgtgtgaaattgttatccgctcacaattccacacaacatacgagccggaagcataaagtgtaaagcctggggtgcctaatgagtgagctaactcacattaattgcgttgcgctcactgcccgctttccagtcgggaaacctgtcgtgccagctgcattaatgaatcggccaacgcgcggggagaggcggtttgcgtattgggcgctcttccgcttcctcgctcactgactcgctgcgctcggtcgttcggctgcggcgagcggtatcagctcactcaaaggcggtaatacggttatccacagaatcaggggataacgcaggaaagaacatgtgagcaaaaggccagcaaaaggccaggaaccgtaaaaaggccgcgttgctggcgtttttccataggctccgcccccctgacgagcatcacaaaaatcgacgctcaagtcagaggtggcgaaacccgacaggactataaagataccaggcgtttccccctggaagctccctcgtgcgctctcctgttccgaccctgccgcttaccggatacctgtccgcctttctcccttcgggaagcgtggcgctttctcatagctcacgctgtaggtatctcagttcggtgtaggtcgttcgctccaagctgggctgtgtgcacgaaccccccgttcagcccgaccgctgcgccttatccggtaactatcgtcttgagtccaacccggtaagacacgacttatcgccactggcagcagccactggtaacaggattagcagagcgaggtatgtaggcggtgctacagagttcttgaagtggtggcctaactacggctacactagaagaacagtatttggtatctgcgctctgctgaagccagttaccttcggaaaaagagttggtagctcttgatccggcaaacaaaccaccgctggtagcggtggtttttttgtttgcaagcagcagattacgcgcagaaaaaaaggatctcaagaagatcctttgatcttttctacggggtctgacgctcagtggaacgaaaactcacgttaagggattttggtcatgagattatcaaaaaggatcttcacctagatccttttaaattaaaaatgaagttttaaatcaatctaaagtatatatgagtaaacttggtctgacagttaccaatgcttaatcagtgaggcacctatctcagcgatctgtctatttcgttcatccatagttgcctgactccccgtcgtgtagataactacgatacgggagggcttaccatctggccccagtgctgcaatgataccgcgagacccacgctcaccggctccagatttatcagcaataaaccagccagccggaagggccgagcgcagaagtggtcctgcaactttatccgcctccatccagtctattaattgttgccgggaagctagagtaagtagttcgccagttaatagtttgcgcaacgttgttgccattgctacaggcatcgtggtgtcacgctcgtcgtttggtatggcttcattcagctccggttcccaacgatcaaggcgagttacatgatcccccatgttgtgcaaaaaagcggttagctccttcggtcctccgatcgttgtcagaagtaagttggccgcagtgttatcactcatggttatggcagcactgcataattctcttactgtcatgccatccgtaagatgcttttctgtgactggtgagtactcaaccaagtcattctgagaatagtgtatgcggcgaccgagttgctcttgcccggcgtcaatacgggataataccgcgccacatagcagaactttaaaagtgctcatcattggaaaacgttcttcggggcgaaaactctcaaggatcttaccgctgttgagatccagttcgatgtaacccactcgtgcacccaactgatcttcagcatcttttactttcaccagcgtttctgggtgagcaaaaacaggaaggcaaaatgccgcaaaaaagggaataagggcgacacggaaatgttgaatactcatactcttcctttttcaatattattgaagcatttatcagggttattgtctcatgagcggatacatatttgaatgtatttagaaaaataaacaaataggggttccgcgcacatttccccgaaaagtgccacctaaattgtaagcgttaatattttgttaaaattcgcgttaaatttttgttaaatcagctcattttttaaccaataggccgaaatcggcaaaatcccttataaatcaaaagaatagaccgagatagggttgagtgttgttccagtttggaacaagagtccactattaaagaacgtggactccaacgtcaaagggcgaaaaaccgtctatcagggcgatggcccactacgtgaaccatcaccctaatcaagttttttggggtcgaggtgccgtaaagcactaaatcggaaccctaaagggagcccccgatttagagcttgacggggaaagccagcgaacgtggcgagagcttgacggggaaagccagcgaacgacggggaaagccagcgaacgtggcgagacttgacggggaaagccaggaacgtggcgagaaagcttgacggggaaagccagcgaacgtggcgagaaaggaagggaagaaagcgaaaggagcgggcgctagggcgctggcaagtgtagcggtcacgctgcgcgtaaccaccacacccgccgcgcttaatgcgccgctacagggcgcgtcccattcgccattcaggctgcgcaactgttgggaagggcgatcggtgcgggcctcttcgctattacgccagctggcgaaagggggatgtgctgcaaggcgattaagttgggtaacgccagggttttcccagtcacgacgttgtaaaacgacggccagtgagcgcgcgtaatacgactcactatagggcgaattgggtaccgggccccccctcgaggtcgacggtatcgataagcttgatatcgaattcctgcagcccgg